European Patent Specification EP 3 480 306 B1, published June 7, 2023. Title: A novel thermostable fructose-6-phosphate-3-epimerase and methods for producing allulose using the same. Applicant: CJ CheilJedang Corporation. The sequence listing filed with the application follows.

SEQUENCE LISTING (8 sequences)

SEQ ID NO: 1 - protein, 221 aa, Artificial Sequence
  fructose-6-phosphate-3-epimerase
MMVKIAASILACDLARLADEVKRVEEHIDMVHFDVMDGHFVPNISFGLPVLKALRKETSLPISVHLMITNPEDYVDRFVEEGADMVAVHYETTPHLHRIVHRIKDLGAKAFVALNPHTPVFLLSEIITDVDGVLVMSVNPGFSGQRFIARSLEKIRSLKKMIRDLGLETEIMVDGGVNEENASILIKNGATILVMGYGIFKNENYVELVRSIKQERGESAG

SEQ ID NO: 2 - DNA, 666 bp, Artificial Sequence
  fructose-6-phosphate-3-epimerase
atgatggtaaagatcgccgcttcaatccttgcgtgtgatcttgcaagactcgccgatgaggtaaaaagggtggaagaacacatagacatggttcacttcgatgtcatggatggacacttcgttccgaacatctcgttcggattgcccgttctcaaagccctgagaaaagaaaccagccttcctataagtgttcatctgatgatcacaaatccagaggactatgtggaccgtttcgtggaagagggagcggacatggtggcggtccactacgagacaacgccgcaccttcacaggatagtgcacaggataaaggatctcggggcgaaggcgttcgtcgccctcaacccacacacaccggtttttctcctgtctgagatcataacggatgtggatggcgtactcgtgatgagtgtgaacccgggcttttctggtcagagattcattgcaaggagtctggaaaaaataaggagtctgaagaagatgataagggatctgggactcgaaacggagatcatggtcgatggtggtgtcaacgaagaaaacgcttctatcttaataaagaacggtgcgacgatccttgtaatggggtacggtatcttcaaaaacgaaaactatgtggaactggtgagatccatcaagcaggaaagaggggaatctgctggctga

SEQ ID NO: 3 - DNA, 34 bp, Artificial Sequence
  forward primer
ggaacatatgatggtaaagatcgccgcttcaatc

SEQ ID NO: 4 - DNA, 27 bp, Artificial Sequence
  reverse primer
catactcgagcttcccctctcctatct

SEQ ID NO: 5 - protein, 270 aa, Artificial Sequence
  polyphosphate-dependent glucokinase
MLAASDSSQHGGKAVTLSPMSVILGIDIGGSGIKGAPVDTATGKLVAERHRIPTPEGAHPDAVKDVVVELVRHFGHAGPVGITFPGIVQHGHTLSAANVDKAWIGLDADTLFTEATGRDVTVINDADAAGLAEARFGAGAGVPGEVLLLTFGTGIGSALIYNGVLVPNTEFGHLYLKGDKHAETWASDRAREQGDLNWKQWAKRVSRYLQYLEGLFSPDLFIIGGGVSKKADKWQPHVATTRTRLVPAALQNEAGIVGAAMVAAQRSQGD

SEQ ID NO: 6 - protein, 253 aa, Artificial Sequence
  polyphosphate-dependent glucokinase
MGRQGMEILGIDIGGSGIKGAPVDVETGQLTAERYRLPTPENALPEEVALVVAQIVEHFQWKGRVGAGFPAAIKHGVAQTAANIHPTWIGLHAGNLFSEKCGCPVSVLNDADAAGLAEMIFGAGKGQKGVVLMITIGTGIGTALFTDGILVPNTELGHIEIRGKDAEQRSSEAARQRKDWTWQQWAKRLNEHLERLEALFWPDLFILGGGAVKNHEKFFPYLKLRTPFVAAKLGNLAGIVGAAWYAHTQETQA

SEQ ID NO: 7 - DNA, 813 bp, Artificial Sequence
  polyphosphate-dependent glucokinase
atgctggcagccagtgacagcagccagcatggcgggaaggctgttacgctatctcccatgagcgtgatcctcgggattgacataggtgggagcggcatcaagggggcccctgtggacacggcaaccgggaagctggtggccgagcgccaccgcatccccacgcccgagggcgcgcacccagacgcggtgaaggacgtggtggttgagctggtgcggcattttgggcatgcggggccagtcggcatcactttccctggcatcgtgcagcacggccataccctgagcgcagccaatgtggataaagcctggattggcctggacgccgacacgctttttactgaggcgaccggtcgcgacgtgaccgtgatcaacgacgcagatgccgcggggctagcggaggcgaggttcggggccggggcaggtgtgccgggcgaggtgttgctgttgacctttgggacaggcatcggcagcgcgctgatctataacggcgtgctggtgcccaacaccgagtttgggcatctgtatctcaagggcgacaagcacgccgagacatgggcgtccgaccgggcccgtgagcagggcgacctgaactggaagcagtgggccaaacgggtcagccggtacctccagtatctggaaggtctcttcagtcccgatctctttatcatcggtgggggcgtgagcaagaaggccgacaagtggcagccgcacgtcgcaacaacacgtacccgcctggtgcccgctgccctccagaacgaggccggaatcgtgggggccgcgatggtggcggcgcagcggtcacagggggactaa

SEQ ID NO: 8 - DNA, 762 bp, Artificial Sequence
  polyphosphate-dependent glucokinase
atggggaggcagggcatggaaattttagggattgatatcggaggatccggcatcaaaggggctccggtggatgtagaaaccggccagttaaccgccgagcgataccgcttacccacccccgaaaatgccttacctgaagaagtggctctggtagttgcccaaattgtcgaacactttcagtggaaaggtcgtgtaggggcaggatttcctgctgccatcaagcacggcgtggcacagacggccgcaaacatccaccctacatggattggacttcatgctggcaaccttttcagcgaaaaatgcggatgtcctgtctcagtgttgaatgatgcggatgctgccggactggcggaaatgatctttggggcaggaaaaggccagaaaggggtggtgctgatgattaccattggcactggcatcgggacagccctgttcaccgatgggatattggtccctaataccgagttgggacatattgaaattcggggcaaagatgccgaacagcgctcttcggaagccgcccgccagcggaaggattggacctggcaacaatgggcaaagcgtctgaatgagcatttggagcgcctggaagccctgttctggcccgatttattcatccttggtggaggggcagtaaaaaatcatgaaaagttcttcccttatctaaaactgcgtactccctttgttgcagcaaaattggggaatctggctgggattgtaggcgcagcgtggtatgctcacacccaggaaacgcaagcctga